European Patent Application EP 4 371 573 A1, published May 22, 2024. Title: Therapeutic agent for inflammatory bowel disease containing anti-IL-18 antibody. Applicant: mAbProtein Co., Ltd. The sequence listing filed with the application follows.

SEQUENCE LISTING (25 sequences)

SEQ ID NO: 1 - protein, 10 aa, Mus musculus
GFSLSSSGMG

SEQ ID NO: 2 - protein, 7 aa, Mus musculus
IWWDDDK

SEQ ID NO: 3 - protein, 15 aa, Mus musculus
TRTRTYSNFGGGMAY

SEQ ID NO: 4 - protein, 11 aa, Mus musculus
QSIAHSNGYTY

SEQ ID NO: 5 - skipped

SEQ ID NO: 6 - protein, 9 aa, Mus musculus
VQGSHVPLT

SEQ ID NO: 7 - protein, 8 aa, Mus musculus
GFSLTSYG

SEQ ID NO: 8 - protein, 7 aa, Mus musculus
IWAGGST

SEQ ID NO: 9 - protein, 11 aa, Mus musculus
ARESSYDAMDY

SEQ ID NO: 10 - protein, 6 aa, Mus musculus
ENVVTY

SEQ ID NO: 11 - skipped

SEQ ID NO: 12 - protein, 9 aa, Mus musculus
GQGYSYPYT

SEQ ID NO: 13 - protein, 105 aa, Mus musculus
SLTCSFSGFSLSSSGMGVGWIRQPSGKGLEWLAHIWWDDDKNYNPGLKSRLTISKDTSKNQVFLKIANVDTADAATYYCTRTRTYSNFGGGMAYWGTRNLSHRLL

SEQ ID NO: 14 - protein, 98 aa, Mus musculus
LGDQASISCRSSQSIAHSNGYTYLEWYLQTPGQSPKLLIYKVSNRFSGVPDRFSGSGSGTDFTLKISRVEAEDLGVYYCVQGSHVPLTFGAGTKLELK

SEQ ID NO: 15 - protein, 100 aa, Mus musculus
LSITCTVSGFSLTSYGVHWVRQPPGKGLEWLGVIWAGGSTNYNSALMSRLSISKDNSKSQVFLKMNSLQTDDTAMYYCARESSYDAMDYWGQGTSVTVSS

SEQ ID NO: 16 - protein, 107 aa, Mus musculus
DIVITQSPKSMSMSVGERVTLTCKASENVVTYVSWYQQKPEQSPKLMIYGASNRYTGVPDRFTGSGSATDFTLTISSVQAEDLADYHCGQGYSYPYTFGGGTKLEIK

SEQ ID NO: 17 - protein, 193 aa, Homo sapiens
MAAEPVEDNCINFVAMKFIDNTLYFIAEDDENLESDYFGKLESKLSVIRNLNDQVLFIDQGNRPLFEDMTDSDCRDNAPRTIFIISMYKDSQPRGMAVTISVKCEKISTLSCENKIISFKEMNPPDNIKDTKSDIIFFQRSVPGHDNKMQFESSSYEGYFLACEKERDLFKLILKKEDELGDRSIMFTVQNED

SEQ ID NO: 18 - protein, 192 aa, Mus musculus
MAAMSEDSCVNFKEMMFIDNTLYFIPEENGDLESDNFGRLHCTTAVIRNINDQVLFVDKRQPVFEDMTDIDQSASEPQTRLIIYMYKDSEVRGLAVTLSVKDSKMSTLSCKNKIISFEEMDPPENIDDIQSDLIFFQKRVPGHNKMEFESSLYEGHFLACQKEDDAFKLILKKKDENGDKSVMFTLTNLHQS

SEQ ID NO: 19 - protein, 10 aa, synthetic construct
  REGION 1..10: note = immunogen
NFGRLHCTTC

SEQ ID NO: 20 - protein, 9 aa, Mus musculus
NFGRLHCTT

SEQ ID NO: 21 - protein, 9 aa, synthetic construct
  REGION 1..9: note = synthetic peptide
AFGRLHCTT

SEQ ID NO: 22 - protein, 9 aa, synthetic construct
  REGION 1..9: note = synthetic peptide
NAGRLHCTT

SEQ ID NO: 23 - protein, 9 aa, synthetic construct
  REGION 1..9: note = synthetic peptide
NFARLHCTT

SEQ ID NO: 24 - protein, 9 aa, synthetic construct
  REGION 1..9: note = synthetic peptide
NFGALHCTT

SEQ ID NO: 25 - skipped